European Patent Application EP 4 610 349 A1, published September 3, 2025. Title: METHOD FOR PRODUCING IMMORTALIZED CELLS. Applicant: KITAYAMA LABES CO.,LTD. Application JP 2022-195145, filed December 1, 2022. The sequence listing filed with the application follows.

SEQUENCE LISTING (21 sequences)

SEQ ID NO: 1 - DNA, 5013 bp, synthetic construct
  source 1..5013: mol_type = other DNA
ctcgacattgattattgactagttattaatagtaatcaattacggggtcattagttcatagcccatatatggagttccgcgttacataacttacggtaaatggcccgcctggctgaccgcccaacgacccccgcccattgacgtcaataatgacgtatgttcccatagtaacgccaatagggactttccattgacgtcaatgggtggagtatttacggtaaactgcccacttggcagtacatcaagtgtatcatatgccaagtacgccccctattgacgtcaatgacggtaaatggcccgcctggcattatgcccagtacatgaccttatgggactttcctacttggcagtacatctacgtattagtcatcgctattaccatggtcgaggtgagccccacgttctgcttcactctccccatctcccccccctccccacccccaattttgtatttatttattttttaattattttgtgcagcgatgggggcggggggggggggggggcgcgcgccaggcggggcggggcggggcgaggggcggggcggggcgaggcggagaggtgcggcggcagccaatcagagcggcgcgctccgaaagtttccttttatggcgaggcggcggcggcggcggccctataaaaagcgaagcgcgcggcgggcgggagtcgctgcgcgctgccttcgccccgtgccccgctccgccgccgcctcgcgccgcccgccccggctctgactgaccgcgttactcccacaggtgagcgggcgggacggcccttctcctccgggctgtaattagcgcttggtttaatgacggcttgtttcttttctgtggctgcgtgaaagccttgaggggctccgggagggccctttgtgcggggggagcggctcggggggtgcgtgcgtgtgtgtgtgcgtggggagcgccgcgtgcggctccgcgctgcccggcggctgtgagcgctgcgggcgcggcgcggggctttgtgcgctccgcagtgtgcgcgaggggagcgcggccgggggcggtgccccgcggtgcggggggggctgcgaggggaacaaaggctgcgtgcggggtgtgtgcgtgggggggtgagcagggggtgtgggcgcgtcggtcgggctgcaaccccccctgcacccccctccccgagttgctgagcacggcccggcttcgggtgcggggctccgtacggggcgtggcgcggggctcgccgtgccgggcggggggtggcggcaggtgggggtgccgggcggggcggggccgcctcgggccggggagggctcgggggaggggcgcggcggcccccggagcgccggcggctgtcgaggcgcggcgagccgcagccattgccttttatggtaatcgtgcgagagggcgcagggacttcctttgtcccaaatctgtgcggagccgaaatctgggaggcgccgccgcaccccctctagcgggcgcggggcgaagcggtgcggcgccggcaggaaggaaatgggcggggagggccttcgtgcgtcgccgcgccgccgtccccttctccctctccagcctcggggctgtccgcggggggacggctgccttcgggggggacggggcagggcggggttcggcttctggcgtgtgaccggcggctctagagcctctgctaaccatgttcatgccttcttctttttcctacagctcctgggcaacgtgctggttattgtgctgtctcatcattttggcaaagccaccatggaacaccagctcctgtgctgcgaagtggaaaccatccgccgcgcgtaccccgatgccaacctcctcaacgaccgggtgctgcgggccatgctgaaggcggaggagacctgcgcgccctcggtgtcctacttcaaatgtgtgcagaaggaggtcctgccgtccatgcggaagatcgtcgccacctggatgctggaggtctgcgaggaacagaagtgcgaggaggaggtcttcccgctggccatgaactacctggaccgcttcctgtcgctggagcccgtgaaaaagagccgcctgcagctgctgggggccacttgcatgttcgtggcctctaagatgaaggagaccatccccctgacggccgagaagctgtgcatctacaccgacaactccatccggcccgaggagctgctgcaaatggagctgctcctggtgaacaagctcaagtggaacctggccgcaatgaccccgcacgatttcattgaacacttcctctccaaaatgccagaggcggaggagaacaaacagatcatccgcaaacacgcgcagaccttcgttgccctctgtgccacagatgtgaagttcatttccaatccgccctccatggtggcagcggggagcgtggtggccgcagtgcaaggcctgaacctgaggagccccaacaacttcctgtcctactaccgcctcacacgcttcctctccagagtgatcaagtgtgacccagactgcctccgggcctgccaggagcagatcgaagccctgctggagtcaagcctgcgccaggcccagcagaacatggaccccaaggccgccgaggaggaggaagaggaggaggaggaggtggacctggcttgcacacccaccgacgtgcgggacgtggacatcggaagcggagctactaacttcagcctgctgaagcaggctggagacgtggaggagaaccctggacctatggcgcacgccgggcgaacagggtacgacaaccgggagatcgtgatgaagtacatccactataagctgtcccagaggggctacgagtgggacgctggggacgcgggcgccgcctccgcgccgggcgtcttctcctcccagcccgcgcccgctgcgccccgggacccggccgccaggacctcgccgccgccgccgccggccgccgcggggcccgcgctcagcccggtgccacctgtggtccacctgaccctccgccaggcgggcgacgacttctcccggcgctaccgccgcgacttcgcggagatgtccagccagctgcacctgacgcccttcaccgcgagggggcgctttgccacggtggtggaggagctcttcagggatggggtgaactgggggaggattgtggccttctttgagttcggtggggtcatgtgtgtggagagcgtcaaccgggagatgtcgcccctggtggacaacatcgccctgtggatgactgagtacctgaaccggcacctgcacacctggatccaggataatggaggctgggatgccttcgtggaactgtacggccccagcgtgcggcctctgtcagacttctcctgggtgtctctgaagactttgttcagcctggccctgataggagcttgcatcaccctcggtgcctacctgggccacaagggaagcggagctactaacttcagcctgctgaagcaggctggagacgtggaggagaaccctggacctatgcccctcaacgtcagcttcgccaccaacaggaactatgacctggactacgactcggtgcagccctatttctactgcgatgaggaggagaacttctaccagcagcagcagcagagcgagctgcagccgccggcgcccagcgaggatatctggaagaaattcgagctgctgcccaccccgcccctgtccccgagccgccgctccggcctctgctcgccctcctacgttgccgtcgcgtccttctcccccaggggagacgacggcggcggcggcggcagcttctccacggctgaccagctggagatggtcaccgagctgctgggcggtgacatggtgaaccagagcttcatctgcgacccggacgacgagaccttcatcaagaacatcatcatccaggactgcatgtggagcggcttctcggccgccgccaagctcgtctcggagaagctggcctcctaccaggctgcgcgcaaggacagcggcagcccgagccccgcccgcggccacggcggctgctccacctccagcctgtacctgcaggacctgagcgccgccgcctccgaatgcatcgacccctcggtggtcttcccctacccactgcacgacagcagctcgcccaagccctgcgcctcgcccgactccagcgccttctccccgtcctcggactctctgctctcctccaacgagtcctctccgcgggccagccctgagcccctggtgctccatgaagagacaccgcccaccaccagcagcgactctgaggaagaacaagaggatgaggaagaaatcgatgtcgtttctgtggaaaagaggcagccctccaccaaaaggtcagggtcaccatctgcagggggccacagcaaacctccacacagcccgctggtcctcaagaggtgccacgtctccacccatcagcacaattacgccgcgcccccatccaccaggaaggactacccagctgccaagcgggccaagttggacagtggccgagtcctgaagcagatcagcaacaatcgcagatgtgccagccccaggtcctcagacaccgaggagaacgacaagaggcggacacacaacgtcttggaacgccagaggagaaatgagctgaaaaggagcttttttgccctgcgtgaccagatcccagagttggaaaacaatgaaaaggcccccaaggtagttatccttaaaaaagccacggcgtacatcctggccgtccaagcagaggagcaaaagctcatttcagagaaggacttgttgcggaaacggcgagaacagttgaaacacaaacttgaacagctacggaactcttgtgcataactcgagtctagagggcccgtttaaacccgctgatcagcctcgactgtgccttctagttgccagccatctgttgtttgcccctcccccgtgccttccttgaccctggaaggtgccactcccactgtcctttcctaataaaatgaggaaattgcatcgcattgtctgagtaggtgtcattctattctggggggtggggtggggcaggacagcaagggggaggattgggaagacaatagcaggcatgctggggatgcggtgggctctatgg

SEQ ID NO: 2 - DNA, 2973 bp, synthetic construct
  source 1..2973: mol_type = other DNA
gtgtgtcagttagggtgtggaaagtccccaggctccccagcaggcagaagtatgcaaagcatgcatctcaattagtcagcaaccaggtgtggaaagtccccaggctccccagcaggcagaagtatgcaaagcatgcatctcaattagtcagcaaccatagtcccgcccctaactccgcccatcccgcccctaactccgcccagttccgcccattctccgccccatggctgactaattttttttatttatgcagaggccgaggccgcctcggcctctgagctattccagaagtagtgaggaggcttttttggaggcctaggcttttgcaaaaagctttgcaaagatggataaagttttaaacagagaggaatctttgcagctaatggaccttctaggtcttgaaaggagtgcctgggggaatattcctctgatgagaaaggcatatttaaaaaaatgcaaggagtttcatcctgataaaggaggagatgaagaaaaaatgaagaaaatgaatactctgtacaagaaaatggaagatggagtaaaatatgctcatcaacctgactttggaggcttctgggatgcaactgaggtatttgcttcttccttaaatcctggtgttgatgcaatgtactgcaaacaatggcctgagtgtgcaaagaaaatgtctgctaactgcatatgcttgctgtgcttactgaggatgaagcatgaaaatagaaaattatacaggaaagatccacttgtgtgggttgattgctactgcttcgattgctttagaatgtggtttggacttgatctttgtgaaggaaccttacttctgtggtgtgacataattggacaaactacctacagagatttaaagctctaaggtaaatataaaatttttaagtgtataatgtgttaaactactgattctaattgtttgtgtattttagattccaacctatggaactgatgaatgggagcagtggtggaatgcctttaatgaggaaaacctgttttgctcagaagaaatgccatctagtgatgatgaggctactgctgactctcaacattctactcctccaaaaaagaagagaaaggtagaagaccccaaggactttccttcagaattgctaagttttttgagtcatgctgtgtttagtaatagaactcttgcttgctttgctatttacaccacaaaggaaaaagctgcactgctatacaagaaaattatggaaaaatattctgtaacctttataagtaggcataacagttataatcataacatactgttttttcttactccacacaggcatagagtgtctgctattaataactatgctcaaaaattgtgtacctttagctttttaatttgtaaaggggttaataaggaatatttgatgtatagtgccttgactagagatccattttctgttattgaggaaagtttgccaggtgggttaaaggagcatgattttaatccagaagaagcagaggaaactaaacaagtgtcctggaagcttgtaacagagtatgcaatggaaacaaaatgtgatgatgtgttgttattgcttgggatgtacttggaatttcagtacagttttgaaatgtgtttaaaatgtattaaaaaagaacagcccagccactataagtaccatgaaaagcattatgcaaatgctgctatatttgctgacagcaaaaaccaaaaaaccatatgccaacaggctgttgatactgttttagctaaaaagcgggttgatagcctacaattaactagagaacaaatgttaacaaacagatttaatgatcttttggataggatggatataatgtttggttctacaggctctgctgacatagaagaatggatggctggagttgcttggctacactgtttgttgcccaaaatggattcagtggtgtatgactttttaaaatgcatggtgtacaacattcctaaaaaaagatactggctgtttaaaggaccaattgatagtggtaaaactacattagcagctgctttgcttgaattatgtggggggaaagctttaaatgttaatttgcccttggacaggctgaactttgagctaggagtagctattgaccagtttttagtagtttttgaggatgtaaagggcactggaggggagtccagagatttgccttcaggtcagggaattaataacctggacaatttaagggattatttggatggcagtgttaaggtaaacttagaaaagaaacacctaaataaaagaactcaaatatttccccctggaatagtcaccatgaatgagtacagtgtgcctaaaacactgcaggccagatttgtaaaacaaatagattttaggcccaaagattatttaaagcattgcctggaacgcagtgagtttttgttagaaaagagaataattcaaagtggcattgctttgcttcttatgttaatttggtacagacctgtggctgagtttgctcaaagtattcagagcagaattgtggagtggaaagagagattggacaaagagtttagtttgtcagtgtatcaaaaaatgaagtttaatgtggctatgggaattggagttttagattggctaagaaacagtgatgatgatgatgaagacagccaggaaaatgctgataaaaatgaagatggtggggagaagaacatggaagactcagggcatgaaacaggcattgattcacagtcccaaggctcatttcaggcccctcagtcctcacagtctgttcatgatcataatcagccataccacatttgtagaggttttacttgctttaaaaaacctcccacacctccccctgaacctgaaacataaaatgaatgcaattgttgttgttaacttgtttattgcagcttataatggttacaaataaagcaatagcatcacaaatttcacaaataaagcatttttttcactgcattctagttgtggtttgtccaaactcatcaatgtatcttatcatgtctggatc

SEQ ID NO: 3 - DNA, 21 bp, synthetic construct
  source 1..21: mol_type = other DNA
ctcaccatggagactgggctg

SEQ ID NO: 4 - DNA, 21 bp, synthetic construct
  source 1..21: mol_type = other DNA
tcatttacccggagagcggga

SEQ ID NO: 5 - DNA, 21 bp, synthetic construct
  source 1..21: mol_type = other DNA
aggcaggacccagcatggaca

SEQ ID NO: 6 - DNA, 20 bp, synthetic construct
  source 1..20: mol_type = other DNA
acagtcacccctattgaagc

SEQ ID NO: 7 - DNA, 1395 bp, Oryctolagus cuniculus
  source 1..1395: mol_type = genomic DNA
atggagactgggctgcgctggcttctcctggtcgctgtgctcaaaggtgtccagtgtcagtcggtggaggagtccgggggtcgcctggtcaagcctgacgaaaccctgacactcacctgcacagtctctggaatcgacctcagtagcgatgcaatgagctgggtccgccaggctccagggaagggactggaatacatcggaatcattagtagtagtggtagcacatactacgcgagctgggcaaaaggccgattcaccatctccagaacctcgaccacggtggatctgaaaatgaccagtccgacaaccgaggacacggccacctatttctgtgccagagtggctgatggtgtttataggggagtagtacttgtgtcgtacttgaacttgtggggcccaggcaccctggtcaccgtctcctcagggcaacctaaggctccatcagtcttcccactggccccctgctgcggggacacacccagctccacggtgaccctgggctgcctggtcaaaggctacctcccggagccagtgaccgtgacctggaactcgggcaccctcaccaatggggtacgcaccttcccgtccgtccggcagtcctcaggcctctactcgctgagcagcgtggtgagcgtgacctcaagcagccagcccgtcacctgcaacgtggcccacccagccaccaacaccaaagtggacaagaccgttgcaccctcgacatgcagcaagcccacgtgcccaccccctgaactcctggggggaccgtctgtcttcatcttccccccaaaacccaaggacaccctcatgatctcacgcacccccgaggtcacatgcgtggtggtggacgtgagccaggatgaccccgaggtgcagttcacatggtacataaacaacgagcaggtgcgcaccgcccggccgccgctacgggagcagcagttcaacagcacgatccgcgtggtcagcaccctccccatcacgcaccaggactggctgaggggcaaggagttcaagtgcaaagtccacaacaaggcactcccggcccccatcgagaaaaccatctccaaagccagagggcagcccctggagccgaaggtctacaccatgggccctccccgggaggagctgagcagcaggtcggtcagcctgacctgcatgatcaacggcttctacccttccgacatctcggtggagtgggagaagaacgggaaggcagaggacaactacaagaccacgccggccgtgctggacagcgacggctcctacttcctctacagcaagctctcagtgcccacgagtgagtggcagcggggcgacgtcttcacctgctccgtgatgcacgaggccttgcacaaccactacacgcagaagtccatctcccgctctccgggtaaatga

SEQ ID NO: 8 - protein, 464 aa, Oryctolagus cuniculus
METGLRWLLLVAVLKGVQCQSVEESGGRLVKPDETLTLTCTVSGIDLSSDAMSWVRQAPGKGLEYIGIISSSGSTYYASWAKGRFTISRTSTTVDLKMTSPTTEDTATYFCARVADGVYRGVVLVSYLNLWGPGTLVTVSSGQPKAPSVFPLAPCCGDTPSSTVTLGCLVKGYLPEPVTVTWNSGTLTNGVRTFPSVRQSSGLYSLSSVVSVTSSSQPVTCNVAHPATNTKVDKTVAPSTCSKPTCPPPELLGGPSVFIFPPKPKDTLMISRTPEVTCVVVDVSQDDPEVQFTWYINNEQVRTARPPLREQQFNSTIRVVSTLPITHQDWLRGKEFKCKVHNKALPAPIEKTISKARGQPLEPKVYTMGPPREELSSRSVSLTCMINGFYPSDISVEWEKNGKAEDNYKTTPAVLDSDGSYFLYSKLSVPTSEWQRGDVFTCSVMHEALHNHYTQKSISRSPGK

SEQ ID NO: 9 - DNA, 714 bp, Oryctolagus cuniculus
  source 1..714: mol_type = genomic DNA
atggacatgagggcccccactcagctgctggggctcctgctgctctggctcccaggtgccacatttgcccaagtgctgacccagactccatcctccgtgtctgcagctgtgggaggcacagtcaccatcaattgccagtccagtccgagtgtttttagtaactacttatcctggtatcagcagaaaccagggcagcctcccaagctccttatctacagggcatccactctggcatctgggggcccatcgcggttcaaaggcagtggatctggggcacagttcactctcaccatcagcgacgtgcagtgtgacgatgctgccacttactactgtgcaggcggttatactactactagtgatggttatgctttcggcggagggaccgaggtggtggtcaaaggtgatccagttgcacctactgtcctcatcttcccaccagctgctgatcaggtggcaactggaacagtcaccatcgtgtgtgtggcgaataaatactttcccgatgtcaccgtcacctgggaggtggatggcaccacccaaacaactggcatcgagaacagtaaaacaccgcagaattctgcagattgtacctacaacctcagcagcactctgacactgaccagcacacagtacaacagccacaaagagtacacctgcaaggtgacccagggcacgacctcagtcgtccagagcttcaataggggtgactgttag

SEQ ID NO: 10 - protein, 237 aa, Oryctolagus cuniculus
MDMRAPTQLLGLLLLWLPGATFAQVLTQTPSSVSAAVGGTVTINCQSSPSVFSNYLSWYQQKPGQPPKLLIYRASTLASGGPSRFKGSGSGAQFTLTISDVQCDDAATYYCAGGYTTTSDGYAFGGGTEVVVKGDPVAPTVLIFPPAADQVATGTVTIVCVANKYFPDVTVTWEVDGTTQTTGIENSKTPQNSADCTYNLSSTLTLTSTQYNSHKEYTCKVTQGTTSVVQSFNRGDC

SEQ ID NO: 11 - DNA, 2682 bp, synthetic construct
  source 1..2682: mol_type = other DNA
ctcgacattgattattgactagttattaatagtaatcaattacggggtcattagttcatagcccatatatggagttccgcgttacataacttacggtaaatggcccgcctggctgaccgcccaacgacccccgcccattgacgtcaataatgacgtatgttcccatagtaacgccaatagggactttccattgacgtcaatgggtggagtatttacggtaaactgcccacttggcagtacatcaagtgtatcatatgccaagtacgccccctattgacgtcaatgacggtaaatggcccgcctggcattatgcccagtacatgaccttatgggactttcctacttggcagtacatctacgtattagtcatcgctattaccatggtcgaggtgagccccacgttctgcttcactctccccatctcccccccctccccacccccaattttgtatttatttattttttaattattttgtgcagcgatgggggcggggggggggggggggcgcgcgccaggcggggcggggcggggcgaggggcggggcggggcgaggcggagaggtgcggcggcagccaatcagagcggcgcgctccgaaagtttccttttatggcgaggcggcggcggcggcggccctataaaaagcgaagcgcgcggcgggcgggagtcgctgcgcgctgccttcgccccgtgccccgctccgccgccgcctcgcgccgcccgccccggctctgactgaccgcgttactcccacaggtgagcgggcgggacggcccttctcctccgggctgtaattagcgcttggtttaatgacggcttgtttcttttctgtggctgcgtgaaagccttgaggggctccgggagggccctttgtgcggggggagcggctcggggggtgcgtgcgtgtgtgtgtgcgtggggagcgccgcgtgcggctccgcgctgcccggcggctgtgagcgctgcgggcgcggcgcggggctttgtgcgctccgcagtgtgcgcgaggggagcgcggccgggggcggtgccccgcggtgcggggggggctgcgaggggaacaaaggctgcgtgcggggtgtgtgcgtgggggggtgagcagggggtgtgggcgcgtcggtcgggctgcaaccccccctgcacccccctccccgagttgctgagcacggcccggcttcgggtgcggggctccgtacggggcgtggcgcggggctcgccgtgccgggcggggggtggcggcaggtgggggtgccgggcggggcggggccgcctcgggccggggagggctcgggggaggggcgcggcggcccccggagcgccggcggctgtcgaggcgcggcgagccgcagccattgccttttatggtaatcgtgcgagagggcgcagggacttcctttgtcccaaatctgtgcggagccgaaatctgggaggcgccgccgcaccccctctagcgggcgcggggcgaagcggtgcggcgccggcaggaaggaaatgggcggggagggccttcgtgcgtcgccgcgccgccgtccccttctccctctccagcctcggggctgtccgcggggggacggctgccttcgggggggacggggcagggcggggttcggcttctggcgtgtgaccggcggctctagagcctctgctaaccatgttcatgccttcttctttttcctacagctcctgggcaacgtgctggttattgtgctgtctcatcattttggcaaagccaccatggcgcacgccgggcgaacagggtacgacaaccgggagatcgtgatgaagtacatccactataagctgtcccagaggggctacgagtgggacgctggggacgcgggcgccgcctccgcgccgggcgtcttctcctcccagcccgcgcccgctgcgccccgggacccggccgccaggacctcgccgccgccgccgccggccgccgcggggcccgcgctcagcccggtgccacctgtggtccacctgaccctccgccaggcgggcgacgacttctcccggcgctaccgccgcgacttcgcggagatgtccagccagctgcacctgacgcccttcaccgcgagggggcgctttgccacggtggtggaggagctcttcagggatggggtgaactgggggaggattgtggccttctttgagttcggtggggtcatgtgtgtggagagcgtcaaccgggagatgtcgcccctggtggacaacatcgccctgtggatgactgagtacctgaaccggcacctgcacacctggatccaggataatggaggctgggatgccttcgtggaactgtacggccccagcgtgcggcctctgtcagacttctcctgggtgtctctgaagactttgttcagcctggccctgataggagcttgcatcaccctcggtgcctacctgggccacaagtaactcgagtctagagggcccgtttaaacccgctgatcagcctcgactgtgccttctagttgccagccatctgttgtttgcccctcccccgtgccttccttgaccctggaaggtgccactcccactgtcctttcctaataaaatgaggaaattgcatcgcattgtctgagtaggtgtcattctattctggggggtggggtggggcaggacagcaagggggaggattgggaagacaatagcaggcatgctggggatgcggtgggctctatgg

SEQ ID NO: 12 - DNA, 2889 bp, synthetic construct
  source 1..2889: mol_type = other DNA
ctcgacattgattattgactagttattaatagtaatcaattacggggtcattagttcatagcccatatatggagttccgcgttacataacttacggtaaatggcccgcctggctgaccgcccaacgacccccgcccattgacgtcaataatgacgtatgttcccatagtaacgccaatagggactttccattgacgtcaatgggtggagtatttacggtaaactgcccacttggcagtacatcaagtgtatcatatgccaagtacgccccctattgacgtcaatgacggtaaatggcccgcctggcattatgcccagtacatgaccttatgggactttcctacttggcagtacatctacgtattagtcatcgctattaccatggtcgaggtgagccccacgttctgcttcactctccccatctcccccccctccccacccccaattttgtatttatttattttttaattattttgtgcagcgatgggggcggggggggggggggggcgcgcgccaggcggggcggggcggggcgaggggcggggcggggcgaggcggagaggtgcggcggcagccaatcagagcggcgcgctccgaaagtttccttttatggcgaggcggcggcggcggcggccctataaaaagcgaagcgcgcggcgggcgggagtcgctgcgcgctgccttcgccccgtgccccgctccgccgccgcctcgcgccgcccgccccggctctgactgaccgcgttactcccacaggtgagcgggcgggacggcccttctcctccgggctgtaattagcgcttggtttaatgacggcttgtttcttttctgtggctgcgtgaaagccttgaggggctccgggagggccctttgtgcggggggagcggctcggggggtgcgtgcgtgtgtgtgtgcgtggggagcgccgcgtgcggctccgcgctgcccggcggctgtgagcgctgcgggcgcggcgcggggctttgtgcgctccgcagtgtgcgcgaggggagcgcggccgggggcggtgccccgcggtgcggggggggctgcgaggggaacaaaggctgcgtgcggggtgtgtgcgtgggggggtgagcagggggtgtgggcgcgtcggtcgggctgcaaccccccctgcacccccctccccgagttgctgagcacggcccggcttcgggtgcggggctccgtacggggcgtggcgcggggctcgccgtgccgggcggggggtggcggcaggtgggggtgccgggcggggcggggccgcctcgggccggggagggctcgggggaggggcgcggcggcccccggagcgccggcggctgtcgaggcgcggcgagccgcagccattgccttttatggtaatcgtgcgagagggcgcagggacttcctttgtcccaaatctgtgcggagccgaaatctgggaggcgccgccgcaccccctctagcgggcgcggggcgaagcggtgcggcgccggcaggaaggaaatgggcggggagggccttcgtgcgtcgccgcgccgccgtccccttctccctctccagcctcggggctgtccgcggggggacggctgccttcgggggggacggggcagggcggggttcggcttctggcgtgtgaccggcggctctagagcctctgctaaccatgttcatgccttcttctttttcctacagctcctgggcaacgtgctggttattgtgctgtctcatcattttggcaaagccaccatggaacaccagctcctgtgctgcgaagtggaaaccatccgccgcgcgtaccccgatgccaacctcctcaacgaccgggtgctgcgggccatgctgaaggcggaggagacctgcgcgccctcggtgtcctacttcaaatgtgtgcagaaggaggtcctgccgtccatgcggaagatcgtcgccacctggatgctggaggtctgcgaggaacagaagtgcgaggaggaggtcttcccgctggccatgaactacctggaccgcttcctgtcgctggagcccgtgaaaaagagccgcctgcagctgctgggggccacttgcatgttcgtggcctctaagatgaaggagaccatccccctgacggccgagaagctgtgcatctacaccgacaactccatccggcccgaggagctgctgcaaatggagctgctcctggtgaacaagctcaagtggaacctggccgcaatgaccccgcacgatttcattgaacacttcctctccaaaatgccagaggcggaggagaacaaacagatcatccgcaaacacgcgcagaccttcgttgccctctgtgccacagatgtgaagttcatttccaatccgccctccatggtggcagcggggagcgtggtggccgcagtgcaaggcctgaacctgaggagccccaacaacttcctgtcctactaccgcctcacacgcttcctctccagagtgatcaagtgtgacccagactgcctccgggcctgccaggagcagatcgaagccctgctggagtcaagcctgcgccaggcccagcagaacatggaccccaaggccgccgaggaggaggaagaggaggaggaggaggtggacctggcttgcacacccaccgacgtgcgggacgtggacatctaactcgagtctagagggcccgtttaaacccgctgatcagcctcgactgtgccttctagttgccagccatctgttgtttgcccctcccccgtgccttccttgaccctggaaggtgccactcccactgtcctttcctaataaaatgaggaaattgcatcgcattgtctgagtaggtgtcattctattctggggggtggggtggggcaggacagcaagggggaggattgggaagacaatagcaggcatgctggggatgcggtgggctctatgg

SEQ ID NO: 13 - DNA, 3318 bp, synthetic construct
  source 1..3318: mol_type = other DNA
ctcgacattgattattgactagttattaatagtaatcaattacggggtcattagttcatagcccatatatggagttccgcgttacataacttacggtaaatggcccgcctggctgaccgcccaacgacccccgcccattgacgtcaataatgacgtatgttcccatagtaacgccaatagggactttccattgacgtcaatgggtggagtatttacggtaaactgcccacttggcagtacatcaagtgtatcatatgccaagtacgccccctattgacgtcaatgacggtaaatggcccgcctggcattatgcccagtacatgaccttatgggactttcctacttggcagtacatctacgtattagtcatcgctattaccatggtcgaggtgagccccacgttctgcttcactctccccatctcccccccctccccacccccaattttgtatttatttattttttaattattttgtgcagcgatgggggcggggggggggggggggcgcgcgccaggcggggcggggcggggcgaggggcggggcggggcgaggcggagaggtgcggcggcagccaatcagagcggcgcgctccgaaagtttccttttatggcgaggcggcggcggcggcggccctataaaaagcgaagcgcgcggcgggcgggagtcgctgcgcgctgccttcgccccgtgccccgctccgccgccgcctcgcgccgcccgccccggctctgactgaccgcgttactcccacaggtgagcgggcgggacggcccttctcctccgggctgtaattagcgcttggtttaatgacggcttgtttcttttctgtggctgcgtgaaagccttgaggggctccgggagggccctttgtgcggggggagcggctcggggggtgcgtgcgtgtgtgtgtgcgtggggagcgccgcgtgcggctccgcgctgcccggcggctgtgagcgctgcgggcgcggcgcggggctttgtgcgctccgcagtgtgcgcgaggggagcgcggccgggggcggtgccccgcggtgcggggggggctgcgaggggaacaaaggctgcgtgcggggtgtgtgcgtgggggggtgagcagggggtgtgggcgcgtcggtcgggctgcaaccccccctgcacccccctccccgagttgctgagcacggcccggcttcgggtgcggggctccgtacggggcgtggcgcggggctcgccgtgccgggcggggggtggcggcaggtgggggtgccgggcggggcggggccgcctcgggccggggagggctcgggggaggggcgcggcggcccccggagcgccggcggctgtcgaggcgcggcgagccgcagccattgccttttatggtaatcgtgcgagagggcgcagggacttcctttgtcccaaatctgtgcggagccgaaatctgggaggcgccgccgcaccccctctagcgggcgcggggcgaagcggtgcggcgccggcaggaaggaaatgggcggggagggccttcgtgcgtcgccgcgccgccgtccccttctccctctccagcctcggggctgtccgcggggggacggctgccttcgggggggacggggcagggcggggttcggcttctggcgtgtgaccggcggctctagagcctctgctaaccatgttcatgccttcttctttttcctacagctcctgggcaacgtgctggttattgtgctgtctcatcattttggcaaagccaccatgcccctcaacgtcagcttcgccaccaacaggaactatgacctggactacgactcggtgcagccctatttctactgcgatgaggaggagaacttctaccagcagcagcagcagagcgagctgcagccgccggcgcccagcgaggatatctggaagaaattcgagctgctgcccaccccgcccctgtccccgagccgccgctccggcctctgctcgccctcctacgttgccgtcgcgtccttctcccccaggggagacgacggcggcggcggcggcagcttctccacggctgaccagctggagatggtcaccgagctgctgggcggtgacatggtgaaccagagcttcatctgcgacccggacgacgagaccttcatcaagaacatcatcatccaggactgcatgtggagcggcttctcggccgccgccaagctcgtctcggagaagctggcctcctaccaggctgcgcgcaaggacagcggcagcccgagccccgcccgcggccacggcggctgctccacctccagcctgtacctgcaggacctgagcgccgccgcctccgaatgcatcgacccctcggtggtcttcccctacccactgcacgacagcagctcgcccaagccctgcgcctcgcccgactccagcgccttctccccgtcctcggactctctgctctcctccaacgagtcctctccgcgggccagccctgagcccctggtgctccatgaagagacaccgcccaccaccagcagcgactctgaggaagaacaagaggatgaggaagaaatcgatgtcgtttctgtggaaaagaggcagccctccaccaaaaggtcagggtcaccatctgcagggggccacagcaaacctccacacagcccgctggtcctcaagaggtgccacgtctccacccatcagcacaattacgccgcgcccccatccaccaggaaggactacccagctgccaagcgggccaagttggacagtggccgagtcctgaagcagatcagcaacaatcgcagatgtgccagccccaggtcctcagacaccgaggagaacgacaagaggcggacacacaacgtcttggaacgccagaggagaaatgagctgaaaaggagcttttttgccctgcgtgaccagatcccagagttggaaaacaatgaaaaggcccccaaggtagttatccttaaaaaagccacggcgtacatcctggccgtccaagcagaggagcaaaagctcatttcagagaaggacttgttgcggaaacggcgagaacagttgaaacacaaacttgaacagctacggaactcttgtgcataactcgagtctagagggcccgtttaaacccgctgatcagcctcgactgtgccttctagttgccagccatctgttgtttgcccctcccccgtgccttccttgaccctggaaggtgccactcccactgtcctttcctaataaaatgaggaaattgcatcgcattgtctgagtaggtgtcattctattctggggggtggggtggggcaggacagcaagggggaggattgggaagacaatagcaggcatgctggggatgcggtgggctctatgg

SEQ ID NO: 14 - DNA, 3633 bp, synthetic construct
  source 1..3633: mol_type = other DNA
ctcgacattgattattgactagttattaatagtaatcaattacggggtcattagttcatagcccatatatggagttccgcgttacataacttacggtaaatggcccgcctggctgaccgcccaacgacccccgcccattgacgtcaataatgacgtatgttcccatagtaacgccaatagggactttccattgacgtcaatgggtggagtatttacggtaaactgcccacttggcagtacatcaagtgtatcatatgccaagtacgccccctattgacgtcaatgacggtaaatggcccgcctggcattatgcccagtacatgaccttatgggactttcctacttggcagtacatctacgtattagtcatcgctattaccatggtcgaggtgagccccacgttctgcttcactctccccatctcccccccctccccacccccaattttgtatttatttattttttaattattttgtgcagcgatgggggcggggggggggggggggcgcgcgccaggcggggcggggcggggcgaggggcggggcggggcgaggcggagaggtgcggcggcagccaatcagagcggcgcgctccgaaagtttccttttatggcgaggcggcggcggcggcggccctataaaaagcgaagcgcgcggcgggcgggagtcgctgcgcgctgccttcgccccgtgccccgctccgccgccgcctcgcgccgcccgccccggctctgactgaccgcgttactcccacaggtgagcgggcgggacggcccttctcctccgggctgtaattagcgcttggtttaatgacggcttgtttcttttctgtggctgcgtgaaagccttgaggggctccgggagggccctttgtgcggggggagcggctcggggggtgcgtgcgtgtgtgtgtgcgtggggagcgccgcgtgcggctccgcgctgcccggcggctgtgagcgctgcgggcgcggcgcggggctttgtgcgctccgcagtgtgcgcgaggggagcgcggccgggggcggtgccccgcggtgcggggggggctgcgaggggaacaaaggctgcgtgcggggtgtgtgcgtgggggggtgagcagggggtgtgggcgcgtcggtcgggctgcaaccccccctgcacccccctccccgagttgctgagcacggcccggcttcgggtgcggggctccgtacggggcgtggcgcggggctcgccgtgccgggcggggggtggcggcaggtgggggtgccgggcggggcggggccgcctcgggccggggagggctcgggggaggggcgcggcggcccccggagcgccggcggctgtcgaggcgcggcgagccgcagccattgccttttatggtaatcgtgcgagagggcgcagggacttcctttgtcccaaatctgtgcggagccgaaatctgggaggcgccgccgcaccccctctagcgggcgcggggcgaagcggtgcggcgccggcaggaaggaaatgggcggggagggccttcgtgcgtcgccgcgccgccgtccccttctccctctccagcctcggggctgtccgcggggggacggctgccttcgggggggacggggcagggcggggttcggcttctggcgtgtgaccggcggctctagagcctctgctaaccatgttcatgccttcttctttttcctacagctcctgggcaacgtgctggttattgtgctgtctcatcattttggcaaagccaccatggaacaccagctcctgtgctgcgaagtggaaaccatccgccgcgcgtaccccgatgccaacctcctcaacgaccgggtgctgcgggccatgctgaaggcggaggagacctgcgcgccctcggtgtcctacttcaaatgtgtgcagaaggaggtcctgccgtccatgcggaagatcgtcgccacctggatgctggaggtctgcgaggaacagaagtgcgaggaggaggtcttcccgctggccatgaactacctggaccgcttcctgtcgctggagcccgtgaaaaagagccgcctgcagctgctgggggccacttgcatgttcgtggcctctaagatgaaggagaccatccccctgacggccgagaagctgtgcatctacaccgacaactccatccggcccgaggagctgctgcaaatggagctgctcctggtgaacaagctcaagtggaacctggccgcaatgaccccgcacgatttcattgaacacttcctctccaaaatgccagaggcggaggagaacaaacagatcatccgcaaacacgcgcagaccttcgttgccctctgtgccacagatgtgaagttcatttccaatccgccctccatggtggcagcggggagcgtggtggccgcagtgcaaggcctgaacctgaggagccccaacaacttcctgtcctactaccgcctcacacgcttcctctccagagtgatcaagtgtgacccagactgcctccgggcctgccaggagcagatcgaagccctgctggagtcaagcctgcgccaggcccagcagaacatggaccccaaggccgccgaggaggaggaagaggaggaggaggaggtggacctggcttgcacacccaccgacgtgcgggacgtggacatcggaagcggagctactaacttcagcctgctgaagcaggctggagacgtggaggagaaccctggacctatggcgcacgccgggcgaacagggtacgacaaccgggagatcgtgatgaagtacatccactataagctgtcccagaggggctacgagtgggacgctggggacgcgggcgccgcctccgcgccgggcgtcttctcctcccagcccgcgcccgctgcgccccgggacccggccgccaggacctcgccgccgccgccgccggccgccgcggggcccgcgctcagcccggtgccacctgtggtccacctgaccctccgccaggcgggcgacgacttctcccggcgctaccgccgcgacttcgcggagatgtccagccagctgcacctgacgcccttcaccgcgagggggcgctttgccacggtggtggaggagctcttcagggatggggtgaactgggggaggattgtggccttctttgagttcggtggggtcatgtgtgtggagagcgtcaaccgggagatgtcgcccctggtggacaacatcgccctgtggatgactgagtacctgaaccggcacctgcacacctggatccaggataatggaggctgggatgccttcgtggaactgtacggccccagcgtgcggcctctgtcagacttctcctgggtgtctctgaagactttgttcagcctggccctgataggagcttgcatcaccctcggtgcctacctgggccacaagtaactcgagtctagagggcccgtttaaacccgctgatcagcctcgactgtgccttctagttgccagccatctgttgtttgcccctcccccgtgccttccttgaccctggaaggtgccactcccactgtcctttcctaataaaatgaggaaattgcatcgcattgtctgagtaggtgtcattctattctggggggtggggtggggcaggacagcaagggggaggattgggaagacaatagcaggcatgctggggatgcggtgggctctatgg

SEQ ID NO: 15 - DNA, 4062 bp, synthetic construct
  source 1..4062: mol_type = other DNA
ctcgacattgattattgactagttattaatagtaatcaattacggggtcattagttcatagcccatatatggagttccgcgttacataacttacggtaaatggcccgcctggctgaccgcccaacgacccccgcccattgacgtcaataatgacgtatgttcccatagtaacgccaatagggactttccattgacgtcaatgggtggagtatttacggtaaactgcccacttggcagtacatcaagtgtatcatatgccaagtacgccccctattgacgtcaatgacggtaaatggcccgcctggcattatgcccagtacatgaccttatgggactttcctacttggcagtacatctacgtattagtcatcgctattaccatggtcgaggtgagccccacgttctgcttcactctccccatctcccccccctccccacccccaattttgtatttatttattttttaattattttgtgcagcgatgggggcggggggggggggggggcgcgcgccaggcggggcggggcggggcgaggggcggggcggggcgaggcggagaggtgcggcggcagccaatcagagcggcgcgctccgaaagtttccttttatggcgaggcggcggcggcggcggccctataaaaagcgaagcgcgcggcgggcgggagtcgctgcgcgctgccttcgccccgtgccccgctccgccgccgcctcgcgccgcccgccccggctctgactgaccgcgttactcccacaggtgagcgggcgggacggcccttctcctccgggctgtaattagcgcttggtttaatgacggcttgtttcttttctgtggctgcgtgaaagccttgaggggctccgggagggccctttgtgcggggggagcggctcggggggtgcgtgcgtgtgtgtgtgcgtggggagcgccgcgtgcggctccgcgctgcccggcggctgtgagcgctgcgggcgcggcgcggggctttgtgcgctccgcagtgtgcgcgaggggagcgcggccgggggcggtgccccgcggtgcggggggggctgcgaggggaacaaaggctgcgtgcggggtgtgtgcgtgggggggtgagcagggggtgtgggcgcgtcggtcgggctgcaaccccccctgcacccccctccccgagttgctgagcacggcccggcttcgggtgcggggctccgtacggggcgtggcgcggggctcgccgtgccgggcggggggtggcggcaggtgggggtgccgggcggggcggggccgcctcgggccggggagggctcgggggaggggcgcggcggcccccggagcgccggcggctgtcgaggcgcggcgagccgcagccattgccttttatggtaatcgtgcgagagggcgcagggacttcctttgtcccaaatctgtgcggagccgaaatctgggaggcgccgccgcaccccctctagcgggcgcggggcgaagcggtgcggcgccggcaggaaggaaatgggcggggagggccttcgtgcgtcgccgcgccgccgtccccttctccctctccagcctcggggctgtccgcggggggacggctgccttcgggggggacggggcagggcggggttcggcttctggcgtgtgaccggcggctctagagcctctgctaaccatgttcatgccttcttctttttcctacagctcctgggcaacgtgctggttattgtgctgtctcatcattttggcaaagccaccatggcgcacgccgggcgaacagggtacgacaaccgggagatcgtgatgaagtacatccactataagctgtcccagaggggctacgagtgggacgctggggacgcgggcgccgcctccgcgccgggcgtcttctcctcccagcccgcgcccgctgcgccccgggacccggccgccaggacctcgccgccgccgccgccggccgccgcggggcccgcgctcagcccggtgccacctgtggtccacctgaccctccgccaggcgggcgacgacttctcccggcgctaccgccgcgacttcgcggagatgtccagccagctgcacctgacgcccttcaccgcgagggggcgctttgccacggtggtggaggagctcttcagggatggggtgaactgggggaggattgtggccttctttgagttcggtggggtcatgtgtgtggagagcgtcaaccgggagatgtcgcccctggtggacaacatcgccctgtggatgactgagtacctgaaccggcacctgcacacctggatccaggataatggaggctgggatgccttcgtggaactgtacggccccagcgtgcggcctctgtcagacttctcctgggtgtctctgaagactttgttcagcctggccctgataggagcttgcatcaccctcggtgcctacctgggccacaagggaagcggagctactaacttcagcctgctgaagcaggctggagacgtggaggagaaccctggacctatgcccctcaacgtcagcttcgccaccaacaggaactatgacctggactacgactcggtgcagccctatttctactgcgatgaggaggagaacttctaccagcagcagcagcagagcgagctgcagccgccggcgcccagcgaggatatctggaagaaattcgagctgctgcccaccccgcccctgtccccgagccgccgctccggcctctgctcgccctcctacgttgccgtcgcgtccttctcccccaggggagacgacggcggcggcggcggcagcttctccacggctgaccagctggagatggtcaccgagctgctgggcggtgacatggtgaaccagagcttcatctgcgacccggacgacgagaccttcatcaagaacatcatcatccaggactgcatgtggagcggcttctcggccgccgccaagctcgtctcggagaagctggcctcctaccaggctgcgcgcaaggacagcggcagcccgagccccgcccgcggccacggcggctgctccacctccagcctgtacctgcaggacctgagcgccgccgcctccgaatgcatcgacccctcggtggtcttcccctacccactgcacgacagcagctcgcccaagccctgcgcctcgcccgactccagcgccttctccccgtcctcggactctctgctctcctccaacgagtcctctccgcgggccagccctgagcccctggtgctccatgaagagacaccgcccaccaccagcagcgactctgaggaagaacaagaggatgaggaagaaatcgatgtcgtttctgtggaaaagaggcagccctccaccaaaaggtcagggtcaccatctgcagggggccacagcaaacctccacacagcccgctggtcctcaagaggtgccacgtctccacccatcagcacaattacgccgcgcccccatccaccaggaaggactacccagctgccaagcgggccaagttggacagtggccgagtcctgaagcagatcagcaacaatcgcagatgtgccagccccaggtcctcagacaccgaggagaacgacaagaggcggacacacaacgtcttggaacgccagaggagaaatgagctgaaaaggagcttttttgccctgcgtgaccagatcccagagttggaaaacaatgaaaaggcccccaaggtagttatccttaaaaaagccacggcgtacatcctggccgtccaagcagaggagcaaaagctcatttcagagaaggacttgttgcggaaacggcgagaacagttgaaacacaaacttgaacagctacggaactcttgtgcataactcgagtctagagggcccgtttaaacccgctgatcagcctcgactgtgccttctagttgccagccatctgttgtttgcccctcccccgtgccttccttgaccctggaaggtgccactcccactgtcctttcctaataaaatgaggaaattgcatcgcattgtctgagtaggtgtcattctattctggggggtggggtggggcaggacagcaagggggaggattgggaagacaatagcaggcatgctggggatgcggtgggctctatgg

SEQ ID NO: 16 - DNA, 4269 bp, synthetic construct
  source 1..4269: mol_type = other DNA
ctcgacattgattattgactagttattaatagtaatcaattacggggtcattagttcatagcccatatatggagttccgcgttacataacttacggtaaatggcccgcctggctgaccgcccaacgacccccgcccattgacgtcaataatgacgtatgttcccatagtaacgccaatagggactttccattgacgtcaatgggtggagtatttacggtaaactgcccacttggcagtacatcaagtgtatcatatgccaagtacgccccctattgacgtcaatgacggtaaatggcccgcctggcattatgcccagtacatgaccttatgggactttcctacttggcagtacatctacgtattagtcatcgctattaccatggtcgaggtgagccccacgttctgcttcactctccccatctcccccccctccccacccccaattttgtatttatttattttttaattattttgtgcagcgatgggggcggggggggggggggggcgcgcgccaggcggggcggggcggggcgaggggcggggcggggcgaggcggagaggtgcggcggcagccaatcagagcggcgcgctccgaaagtttccttttatggcgaggcggcggcggcggcggccctataaaaagcgaagcgcgcggcgggcgggagtcgctgcgcgctgccttcgccccgtgccccgctccgccgccgcctcgcgccgcccgccccggctctgactgaccgcgttactcccacaggtgagcgggcgggacggcccttctcctccgggctgtaattagcgcttggtttaatgacggcttgtttcttttctgtggctgcgtgaaagccttgaggggctccgggagggccctttgtgcggggggagcggctcggggggtgcgtgcgtgtgtgtgtgcgtggggagcgccgcgtgcggctccgcgctgcccggcggctgtgagcgctgcgggcgcggcgcggggctttgtgcgctccgcagtgtgcgcgaggggagcgcggccgggggcggtgccccgcggtgcggggggggctgcgaggggaacaaaggctgcgtgcggggtgtgtgcgtgggggggtgagcagggggtgtgggcgcgtcggtcgggctgcaaccccccctgcacccccctccccgagttgctgagcacggcccggcttcgggtgcggggctccgtacggggcgtggcgcggggctcgccgtgccgggcggggggtggcggcaggtgggggtgccgggcggggcggggccgcctcgggccggggagggctcgggggaggggcgcggcggcccccggagcgccggcggctgtcgaggcgcggcgagccgcagccattgccttttatggtaatcgtgcgagagggcgcagggacttcctttgtcccaaatctgtgcggagccgaaatctgggaggcgccgccgcaccccctctagcgggcgcggggcgaagcggtgcggcgccggcaggaaggaaatgggcggggagggccttcgtgcgtcgccgcgccgccgtccccttctccctctccagcctcggggctgtccgcggggggacggctgccttcgggggggacggggcagggcggggttcggcttctggcgtgtgaccggcggctctagagcctctgctaaccatgttcatgccttcttctttttcctacagctcctgggcaacgtgctggttattgtgctgtctcatcattttggcaaagccaccatggaacaccagctcctgtgctgcgaagtggaaaccatccgccgcgcgtaccccgatgccaacctcctcaacgaccgggtgctgcgggccatgctgaaggcggaggagacctgcgcgccctcggtgtcctacttcaaatgtgtgcagaaggaggtcctgccgtccatgcggaagatcgtcgccacctggatgctggaggtctgcgaggaacagaagtgcgaggaggaggtcttcccgctggccatgaactacctggaccgcttcctgtcgctggagcccgtgaaaaagagccgcctgcagctgctgggggccacttgcatgttcgtggcctctaagatgaaggagaccatccccctgacggccgagaagctgtgcatctacaccgacaactccatccggcccgaggagctgctgcaaatggagctgctcctggtgaacaagctcaagtggaacctggccgcaatgaccccgcacgatttcattgaacacttcctctccaaaatgccagaggcggaggagaacaaacagatcatccgcaaacacgcgcagaccttcgttgccctctgtgccacagatgtgaagttcatttccaatccgccctccatggtggcagcggggagcgtggtggccgcagtgcaaggcctgaacctgaggagccccaacaacttcctgtcctactaccgcctcacacgcttcctctccagagtgatcaagtgtgacccagactgcctccgggcctgccaggagcagatcgaagccctgctggagtcaagcctgcgccaggcccagcagaacatggaccccaaggccgccgaggaggaggaagaggaggaggaggaggtggacctggcttgcacacccaccgacgtgcgggacgtggacatcggaagcggagctactaacttcagcctgctgaagcaggctggagacgtggaggagaaccctggacctatgcccctcaacgtcagcttcgccaccaacaggaactatgacctggactacgactcggtgcagccctatttctactgcgatgaggaggagaacttctaccagcagcagcagcagagcgagctgcagccgccggcgcccagcgaggatatctggaagaaattcgagctgctgcccaccccgcccctgtccccgagccgccgctccggcctctgctcgccctcctacgttgccgtcgcgtccttctcccccaggggagacgacggcggcggcggcggcagcttctccacggctgaccagctggagatggtcaccgagctgctgggcggtgacatggtgaaccagagcttcatctgcgacccggacgacgagaccttcatcaagaacatcatcatccaggactgcatgtggagcggcttctcggccgccgccaagctcgtctcggagaagctggcctcctaccaggctgcgcgcaaggacagcggcagcccgagccccgcccgcggccacggcggctgctccacctccagcctgtacctgcaggacctgagcgccgccgcctccgaatgcatcgacccctcggtggtcttcccctacccactgcacgacagcagctcgcccaagccctgcgcctcgcccgactccagcgccttctccccgtcctcggactctctgctctcctccaacgagtcctctccgcgggccagccctgagcccctggtgctccatgaagagacaccgcccaccaccagcagcgactctgaggaagaacaagaggatgaggaagaaatcgatgtcgtttctgtggaaaagaggcagccctccaccaaaaggtcagggtcaccatctgcagggggccacagcaaacctccacacagcccgctggtcctcaagaggtgccacgtctccacccatcagcacaattacgccgcgcccccatccaccaggaaggactacccagctgccaagcgggccaagttggacagtggccgagtcctgaagcagatcagcaacaatcgcagatgtgccagccccaggtcctcagacaccgaggagaacgacaagaggcggacacacaacgtcttggaacgccagaggagaaatgagctgaaaaggagcttttttgccctgcgtgaccagatcccagagttggaaaacaatgaaaaggcccccaaggtagttatccttaaaaaagccacggcgtacatcctggccgtccaagcagaggagcaaaagctcatttcagagaaggacttgttgcggaaacggcgagaacagttgaaacacaaacttgaacagctacggaactcttgtgcataactcgagtctagagggcccgtttaaacccgctgatcagcctcgactgtgccttctagttgccagccatctgttgtttgcccctcccccgtgccttccttgaccctggaaggtgccactcccactgtcctttcctaataaaatgaggaaattgcatcgcattgtctgagtaggtgtcattctattctggggggtggggtggggcaggacagcaagggggaggattgggaagacaatagcaggcatgctggggatgcggtgggctctatgg

SEQ ID NO: 17 - DNA, 5034 bp, synthetic construct
  source 1..5034: mol_type = other DNA
ctcgacattgattattgactagttattaatagtaatcaattacggggtcattagttcatagcccatatatggagttccgcgttacataacttacggtaaatggcccgcctggctgaccgcccaacgacccccgcccattgacgtcaataatgacgtatgttcccatagtaacgccaatagggactttccattgacgtcaatgggtggagtatttacggtaaactgcccacttggcagtacatcaagtgtatcatatgccaagtacgccccctattgacgtcaatgacggtaaatggcccgcctggcattatgcccagtacatgaccttatgggactttcctacttggcagtacatctacgtattagtcatcgctattaccatggtcgaggtgagccccacgttctgcttcactctccccatctcccccccctccccacccccaattttgtatttatttattttttaattattttgtgcagcgatgggggcggggggggggggggggcgcgcgccaggcggggcggggcggggcgaggggcggggcggggcgaggcggagaggtgcggcggcagccaatcagagcggcgcgctccgaaagtttccttttatggcgaggcggcggcggcggcggccctataaaaagcgaagcgcgcggcgggcgggagtcgctgcgcgctgccttcgccccgtgccccgctccgccgccgcctcgcgccgcccgccccggctctgactgaccgcgttactcccacaggtgagcgggcgggacggcccttctcctccgggctgtaattagcgcttggtttaatgacggcttgtttcttttctgtggctgcgtgaaagccttgaggggctccgggagggccctttgtgcggggggagcggctcggggggtgcgtgcgtgtgtgtgtgcgtggggagcgccgcgtgcggctccgcgctgcccggcggctgtgagcgctgcgggcgcggcgcggggctttgtgcgctccgcagtgtgcgcgaggggagcgcggccgggggcggtgccccgcggtgcggggggggctgcgaggggaacaaaggctgcgtgcggggtgtgtgcgtgggggggtgagcagggggtgtgggcgcgtcggtcgggctgcaaccccccctgcacccccctccccgagttgctgagcacggcccggcttcgggtgcggggctccgtacggggcgtggcgcggggctcgccgtgccgggcggggggtggcggcaggtgggggtgccgggcggggcggggccgcctcgggccggggagggctcgggggaggggcgcggcggcccccggagcgccggcggctgtcgaggcgcggcgagccgcagccattgccttttatggtaatcgtgcgagagggcgcagggacttcctttgtcccaaatctgtgcggagccgaaatctgggaggcgccgccgcaccccctctagcgggcgcggggcgaagcggtgcggcgccggcaggaaggaaatgggcggggagggccttcgtgcgtcgccgcgccgccgtccccttctccctctccagcctcggggctgtccgcggggggacggctgccttcgggggggacggggcagggcggggttcggcttctggcgtgtgaccggcggctctagagcctctgctaaccatgttcatgccttcttctttttcctacagctcctgggcaacgtgctggttattgtgctgtctcatcattttggcaaagccaccatggaacaccagctcctgtgctgcgaagtggaaaccatccgccgcgcgtaccccgatgccaacctcctcaacgaccgggtgctgcgggccatgctgaaggcggaggagacctgcgcgccctcggtgtcctacttcaaatgtgtgcagaaggaggtcctgccgtccatgcggaagatcgtcgccacctggatgctggaggtctgcgaggaacagaagtgcgaggaggaggtcttcccgctggccatgaactacctggaccgcttcctgtcgctggagcccgtgaaaaagagccgcctgcagctgctgggggccacttgcatgttcgtggcctctaagatgaaggagaccatccccctgacggccgagaagctgtgcatctacaccgacaactccatccggcccgaggagctgctgcaaatggagctgctcctggtgaacaagctcaagtggaacctggccgcaatgaccccgcacgatttcattgaacacttcctctccaaaatgccagaggcggaggagaacaaacagatcatccgcaaacacgcgcagaccttcgttgccctctgtgccacagatgtgaagttcatttccaatccgccctccatggtggcagcggggagcgtggtggccgcagtgcaaggcctgaacctgaggagccccaacaacttcctgtcctactaccgcctcacacgcttcctctccagagtgatcaagtgtgacccagactgcctccgggcctgccaggagcagatcgaagccctgctggagtcaagcctgcgccaggcccagcagaacatggaccccaaggccgccgaggaggaggaagaggaggaggaggaggtggacctggcttgcacacccaccgacgtgcgggacgtggacatcggaagcggagctactaacttcagcctgctgaagcaggctggagacgtggaggagaaccctggacctatgtctcagagcaaccgggagctggtggttgactttctctcctacaagctttcccagaaaggatacagctggagtcagtttagtgatgtggaagagaacaggactgaggccccagaagggactgaatcggagatggagacccccagtgccatcaatggcaacccatcctggcacctggcagacagccccgcggtgaatggagccactggccacagcagcagtttggatgcccgggaggtgatccccatggcagcagtaaagcaagcgctgagggaggcaggcgacgagtttgaactgcggtaccggcgggcattcagtgacctgacatcccagctccacatcaccccagggacagcatatcagagctttgaacaggtagtgaatgaactcttccgggatggggtaaactggggtcgcattgtggcctttttctccttcggcggggcactgtgcgtggaaagcgtagacaaggagatgcaggtattggtgagtcggatcgcagcttggatggccacttacctgaatgaccacctagagccttggatccaggagaacggcggctgggatacttttgtggaactctatgggaacaatgcagcagccgagagccgaaagggccaggaacgcttcaaccgctggttcctgacgggcatgactgtggccggcgtggttctgctgggctcactcttcagtcggaaaggaagcggagctactaacttcagcctgctgaagcaggctggagacgtggaggagaaccctggacctatgcccctcaacgtcagcttcgccaccaacaggaactatgacctggactacgactcggtgcagccctatttctactgcgatgaggaggagaacttctaccagcagcagcagcagagcgagctgcagccgccggcgcccagcgaggatatctggaagaaattcgagctgctgcccaccccgcccctgtccccgagccgccgctccggcctctgctcgccctcctacgttgccgtcgcgtccttctcccccaggggagacgacggcggcggcggcggcagcttctccacggctgaccagctggagatggtcaccgagctgctgggcggtgacatggtgaaccagagcttcatctgcgacccggacgacgagaccttcatcaagaacatcatcatccaggactgcatgtggagcggcttctcggccgccgccaagctcgtctcggagaagctggcctcctaccaggctgcgcgcaaggacagcggcagcccgagccccgcccgcggccacggcggctgctccacctccagcctgtacctgcaggacctgagcgccgccgcctccgaatgcatcgacccctcggtggtcttcccctacccactgcacgacagcagctcgcccaagccctgcgcctcgcccgactccagcgccttctccccgtcctcggactctctgctctcctccaacgagtcctctccgcgggccagccctgagcccctggtgctccatgaagagacaccgcccaccaccagcagcgactctgaggaagaacaagaggatgaggaagaaatcgatgtcgtttctgtggaaaagaggcagccctccaccaaaaggtcagggtcaccatctgcagggggccacagcaaacctccacacagcccgctggtcctcaagaggtgccacgtctccacccatcagcacaattacgccgcgcccccatccaccaggaaggactacccagctgccaagcgggccaagttggacagtggccgagtcctgaagcagatcagcaacaatcgcagatgtgccagccccaggtcctcagacaccgaggagaacgacaagaggcggacacacaacgtcttggaacgccagaggagaaatgagctgaaaaggagcttttttgccctgcgtgaccagatcccagagttggaaaacaatgaaaaggcccccaaggtagttatccttaaaaaagccacggcgtacatcctggccgtccaagcagaggagcaaaagctcatttcagagaaggacttgttgcggaaacggcgagaacagttgaaacacaaacttgaacagctacggaactcttgtgcataactcgagtctagagggcccgtttaaacccgctgatcagcctcgactgtgccttctagttgccagccatctgttgtttgcccctcccccgtgccttccttgaccctggaaggtgccactcccactgtcctttcctaataaaatgaggaaattgcatcgcattgtctgagtaggtgtcattctattctggggggtggggtggggcaggacagcaagggggaggattgggaagacaatagcaggcatgctggggatgcggtgggctctatgg

SEQ ID NO: 18 - DNA, 5004 bp, synthetic construct
  source 1..5004: mol_type = other DNA
ctcgacattgattattgactagttattaatagtaatcaattacggggtcattagttcatagcccatatatggagttccgcgttacataacttacggtaaatggcccgcctggctgaccgcccaacgacccccgcccattgacgtcaataatgacgtatgttcccatagtaacgccaatagggactttccattgacgtcaatgggtggagtatttacggtaaactgcccacttggcagtacatcaagtgtatcatatgccaagtacgccccctattgacgtcaatgacggtaaatggcccgcctggcattatgcccagtacatgaccttatgggactttcctacttggcagtacatctacgtattagtcatcgctattaccatggtcgaggtgagccccacgttctgcttcactctccccatctcccccccctccccacccccaattttgtatttatttattttttaattattttgtgcagcgatgggggcggggggggggggggggcgcgcgccaggcggggcggggcggggcgaggggcggggcggggcgaggcggagaggtgcggcggcagccaatcagagcggcgcgctccgaaagtttccttttatggcgaggcggcggcggcggcggccctataaaaagcgaagcgcgcggcgggcgggagtcgctgcgcgctgccttcgccccgtgccccgctccgccgccgcctcgcgccgcccgccccggctctgactgaccgcgttactcccacaggtgagcgggcgggacggcccttctcctccgggctgtaattagcgcttggtttaatgacggcttgtttcttttctgtggctgcgtgaaagccttgaggggctccgggagggccctttgtgcggggggagcggctcggggggtgcgtgcgtgtgtgtgtgcgtggggagcgccgcgtgcggctccgcgctgcccggcggctgtgagcgctgcgggcgcggcgcggggctttgtgcgctccgcagtgtgcgcgaggggagcgcggccgggggcggtgccccgcggtgcggggggggctgcgaggggaacaaaggctgcgtgcggggtgtgtgcgtgggggggtgagcagggggtgtgggcgcgtcggtcgggctgcaaccccccctgcacccccctccccgagttgctgagcacggcccggcttcgggtgcggggctccgtacggggcgtggcgcggggctcgccgtgccgggcggggggtggcggcaggtgggggtgccgggcggggcggggccgcctcgggccggggagggctcgggggaggggcgcggcggcccccggagcgccggcggctgtcgaggcgcggcgagccgcagccattgccttttatggtaatcgtgcgagagggcgcagggacttcctttgtcccaaatctgtgcggagccgaaatctgggaggcgccgccgcaccccctctagcgggcgcggggcgaagcggtgcggcgccggcaggaaggaaatgggcggggagggccttcgtgcgtcgccgcgccgccgtccccttctccctctccagcctcggggctgtccgcggggggacggctgccttcgggggggacggggcagggcggggttcggcttctggcgtgtgaccggcggctctagagcctctgctaaccatgttcatgccttcttctttttcctacagctcctgggcaacgtgctggttattgtgctgtctcatcattttggcaaagccaccatggagctgctgtgttgcgaaggcacccggcacgcgccccgggccgggccggacccgcggctgctgggggaccagcgtgtcctgcagagcctgctccgcctggaggagcgctacgtaccccgcgcctcctacttccagtgcgtgcagcgggagatcaagccgcacatgcggaagatgctggcttactggatgctggaggtatgtgaggagcagcgctgtgaggaggaagtcttccccctggccatgaactacctggatcgctacctgtcttgcgtccccacccgaaaggcgcagttgcagctcctgggtgcggtctgcatgctgctggcctccaagctgcgcgagaccacgcccctgaccatcgaaaaactgtgcatctacaccgaccacgctgtctctccccgccagttgcgggactgggaggtgctggtcctagggaagctcaagtgggacctggctgctgtgattgcacatgatttcctggccttcattctgcaccggctctctctgccccgtgaccgacaggccttggtcaaaaagcatgcccagacctttttggccctctgtgctacagattatacctttgccatgtacccgccatccatgatcgccacgggcagcattggggctgcagtgcaaggcctgggtgcctgctccatgtccggggatgagctcacagagctgctggcagggatcactggcactgaagtggactgcctgcgggcctgtcaggagcagatcgaagctgcactcagggagagcctcagggaagcctctcagaccagctccagcccagcgcccaaagccccccggggctccagcagccaagggcccagccagaccagcactcctacagatgtcacagccatacacctgggaagcggagctactaacttcagcctgctgaagcaggctggagacgtggaggagaaccctggacctatggcgcacgccgggcgaacagggtacgacaaccgggagatcgtgatgaagtacatccactataagctgtcccagaggggctacgagtgggacgctggggacgcgggcgccgcctccgcgccgggcgtcttctcctcccagcccgcgcccgctgcgccccgggacccggccgccaggacctcgccgccgccgccgccggccgccgcggggcccgcgctcagcccggtgccacctgtggtccacctgaccctccgccaggcgggcgacgacttctcccggcgctaccgccgcgacttcgcggagatgtccagccagctgcacctgacgcccttcaccgcgagggggcgctttgccacggtggtggaggagctcttcagggatggggtgaactgggggaggattgtggccttctttgagttcggtggggtcatgtgtgtggagagcgtcaaccgggagatgtcgcccctggtggacaacatcgccctgtggatgactgagtacctgaaccggcacctgcacacctggatccaggataatggaggctgggatgccttcgtggaactgtacggccccagcgtgcggcctctgtcagacttctcctgggtgtctctgaagactttgttcagcctggccctgataggagcttgcatcaccctcggtgcctacctgggccacaagggaagcggagctactaacttcagcctgctgaagcaggctggagacgtggaggagaaccctggacctatgcccctcaacgtcagcttcgccaccaacaggaactatgacctggactacgactcggtgcagccctatttctactgcgatgaggaggagaacttctaccagcagcagcagcagagcgagctgcagccgccggcgcccagcgaggatatctggaagaaattcgagctgctgcccaccccgcccctgtccccgagccgccgctccggcctctgctcgccctcctacgttgccgtcgcgtccttctcccccaggggagacgacggcggcggcggcggcagcttctccacggctgaccagctggagatggtcaccgagctgctgggcggtgacatggtgaaccagagcttcatctgcgacccggacgacgagaccttcatcaagaacatcatcatccaggactgcatgtggagcggcttctcggccgccgccaagctcgtctcggagaagctggcctcctaccaggctgcgcgcaaggacagcggcagcccgagccccgcccgcggccacggcggctgctccacctccagcctgtacctgcaggacctgagcgccgccgcctccgaatgcatcgacccctcggtggtcttcccctacccactgcacgacagcagctcgcccaagccctgcgcctcgcccgactccagcgccttctccccgtcctcggactctctgctctcctccaacgagtcctctccgcgggccagccctgagcccctggtgctccatgaagagacaccgcccaccaccagcagcgactctgaggaagaacaagaggatgaggaagaaatcgatgtcgtttctgtggaaaagaggcagccctccaccaaaaggtcagggtcaccatctgcagggggccacagcaaacctccacacagcccgctggtcctcaagaggtgccacgtctccacccatcagcacaattacgccgcgcccccatccaccaggaaggactacccagctgccaagcgggccaagttggacagtggccgagtcctgaagcagatcagcaacaatcgcagatgtgccagccccaggtcctcagacaccgaggagaacgacaagaggcggacacacaacgtcttggaacgccagaggagaaatgagctgaaaaggagcttttttgccctgcgtgaccagatcccagagttggaaaacaatgaaaaggcccccaaggtagttatccttaaaaaagccacggcgtacatcctggccgtccaagcagaggagcaaaagctcatttcagagaaggacttgttgcggaaacggcgagaacagttgaaacacaaacttgaacagctacggaactcttgtgcataactcgagtctagagggcccgtttaaacccgctgatcagcctcgactgtgccttctagttgccagccatctgttgtttgcccctcccccgtgccttccttgaccctggaaggtgccactcccactgtcctttcctaataaaatgaggaaattgcatcgcattgtctgagtaggtgtcattctattctggggggtggggtggggcaggacagcaagggggaggattgggaagacaatagcaggcatgctggggatgcggtgggctctatgg

SEQ ID NO: 19 - DNA, 4881 bp, synthetic construct
  source 1..4881: mol_type = other DNA
ctcgacattgattattgactagttattaatagtaatcaattacggggtcattagttcatagcccatatatggagttccgcgttacataacttacggtaaatggcccgcctggctgaccgcccaacgacccccgcccattgacgtcaataatgacgtatgttcccatagtaacgccaatagggactttccattgacgtcaatgggtggagtatttacggtaaactgcccacttggcagtacatcaagtgtatcatatgccaagtacgccccctattgacgtcaatgacggtaaatggcccgcctggcattatgcccagtacatgaccttatgggactttcctacttggcagtacatctacgtattagtcatcgctattaccatggtcgaggtgagccccacgttctgcttcactctccccatctcccccccctccccacccccaattttgtatttatttattttttaattattttgtgcagcgatgggggcggggggggggggggggcgcgcgccaggcggggcggggcggggcgaggggcggggcggggcgaggcggagaggtgcggcggcagccaatcagagcggcgcgctccgaaagtttccttttatggcgaggcggcggcggcggcggccctataaaaagcgaagcgcgcggcgggcgggagtcgctgcgcgctgccttcgccccgtgccccgctccgccgccgcctcgcgccgcccgccccggctctgactgaccgcgttactcccacaggtgagcgggcgggacggcccttctcctccgggctgtaattagcgcttggtttaatgacggcttgtttcttttctgtggctgcgtgaaagccttgaggggctccgggagggccctttgtgcggggggagcggctcggggggtgcgtgcgtgtgtgtgtgcgtggggagcgccgcgtgcggctccgcgctgcccggcggctgtgagcgctgcgggcgcggcgcggggctttgtgcgctccgcagtgtgcgcgaggggagcgcggccgggggcggtgccccgcggtgcggggggggctgcgaggggaacaaaggctgcgtgcggggtgtgtgcgtgggggggtgagcagggggtgtgggcgcgtcggtcgggctgcaaccccccctgcacccccctccccgagttgctgagcacggcccggcttcgggtgcggggctccgtacggggcgtggcgcggggctcgccgtgccgggcggggggtggcggcaggtgggggtgccgggcggggcggggccgcctcgggccggggagggctcgggggaggggcgcggcggcccccggagcgccggcggctgtcgaggcgcggcgagccgcagccattgccttttatggtaatcgtgcgagagggcgcagggacttcctttgtcccaaatctgtgcggagccgaaatctgggaggcgccgccgcaccccctctagcgggcgcggggcgaagcggtgcggcgccggcaggaaggaaatgggcggggagggccttcgtgcgtcgccgcgccgccgtccccttctccctctccagcctcggggctgtccgcggggggacggctgccttcgggggggacggggcagggcggggttcggcttctggcgtgtgaccggcggctctagagcctctgctaaccatgttcatgccttcttctttttcctacagctcctgggcaacgtgctggttattgtgctgtctcatcattttggcaaagccaccatggaacaccagctcctgtgctgcgaagtggaaaccatccgccgcgcgtaccccgatgccaacctcctcaacgaccgggtgctgcgggccatgctgaaggcggaggagacctgcgcgccctcggtgtcctacttcaaatgtgtgcagaaggaggtcctgccgtccatgcggaagatcgtcgccacctggatgctggaggtctgcgaggaacagaagtgcgaggaggaggtcttcccgctggccatgaactacctggaccgcttcctgtcgctggagcccgtgaaaaagagccgcctgcagctgctgggggccacttgcatgttcgtggcctctaagatgaaggagaccatccccctgacggccgagaagctgtgcatctacaccgacaactccatccggcccgaggagctgctgcaaatggagctgctcctggtgaacaagctcaagtggaacctggccgcaatgaccccgcacgatttcattgaacacttcctctccaaaatgccagaggcggaggagaacaaacagatcatccgcaaacacgcgcagaccttcgttgccctctgtgccacagatgtgaagttcatttccaatccgccctccatggtggcagcggggagcgtggtggccgcagtgcaaggcctgaacctgaggagccccaacaacttcctgtcctactaccgcctcacacgcttcctctccagagtgatcaagtgtgacccagactgcctccgggcctgccaggagcagatcgaagccctgctggagtcaagcctgcgccaggcccagcagaacatggaccccaaggccgccgaggaggaggaagaggaggaggaggaggtggacctggcttgcacacccaccgacgtgcgggacgtggacatcggaagcggagctactaacttcagcctgctgaagcaggctggagacgtggaggagaaccctggacctatggcgcacgccgggcgaacagggtacgacaaccgggagatcgtgatgaagtacatccactataagctgtcccagaggggctacgagtgggacgctggggacgcgggcgccgcctccgcgccgggcgtcttctcctcccagcccgcgcccgctgcgccccgggacccggccgccaggacctcgccgccgccgccgccggccgccgcggggcccgcgctcagcccggtgccacctgtggtccacctgaccctccgccaggcgggcgacgacttctcccggcgctaccgccgcgacttcgcggagatgtccagccagctgcacctgacgcccttcaccgcgagggggcgctttgccacggtggtggaggagctcttcagggatggggtgaactgggggaggattgtggccttctttgagttcggtggggtcatgtgtgtggagagcgtcaaccgggagatgtcgcccctggtggacaacatcgccctgtggatgactgagtacctgaaccggcacctgcacacctggatccaggataatggaggctgggatgccttcgtggaactgtacggccccagcgtgcggcctctgtcagacttctcctgggtgtctctgaagactttgttcagcctggccctgataggagcttgcatcaccctcggtgcctacctgggccacaagggaagcggagctactaacttcagcctgctgaagcaggctggagacgtggaggagaaccctggacctatgtgcgtgtgtgctggctgccgggctgccccgagccggcggggagccggtccgctccaggtggcgggcggctggagcgagggagcggacatggactacgactcgtaccagcactatttctacgactatgactgcggggaggatttctaccgctccacggcgcccagcgaggacatctggaagaaattcgagctggtgccatcgccccccacgtcgccgccctggggcttgggtcccggcgcaggggacccggcccccgggattggtcccccggagccgtggcccggagggtgcaccggagacgaagcggaatcccggggccactcgaaaggctggggcaggaactacgcctccatcatacgccgtgactgcatgtggagcggcttctcggcccgggaacggctggagagagctgtgagcgaccggctcgctcctggcgcgccccgggggaacccgcccaaggcgtccgccgccccggactgcactcccagcctcgaagccggcaacccggcgcccgccgccccctgtccgctgggcgaacccaagacccaggcctgctccgggtccgagagcccaagcgactcggagaatgaagaaattgatgttgtgacagtagagaagaggcagtctctgggtattcggaagccggtcaccatcacggtgcgagcagaccccctggatccctgcatgaagcatttccacatctccatccatcagcaacagcacaactatgctgcccgttttcctccagaaagctgctcccaagaagaggcttcagagaggggtccccaagaagaggttctggagagagatgctgcaggggaaaaggaagatgaggaggatgaagagattgtgagtcccccacctgtagaaagtgaggctgcccagtcctgccaccccaaacctgtcagttctgatactgaggatgtgaccaagaggaagaatcacaacttcctggagcgcaagaggcggaatgacctgcgttcgcgattcttggcgctgagggaccaggtgcccaccctggccagctgctccaaggcccccaaagtagtgatcctaagcaaggccttggaatacttgcaagccctggtgggggctgagaagaggatggctacagagaaaagacagctccgatgccggcagcagcagttgcagaaaagaattgcatacctcactggctactaactcgagtctagagggcccgtttaaacccgctgatcagcctcgactgtgccttctagttgccagccatctgttgtttgcccctcccccgtgccttccttgaccctggaaggtgccactcccactgtcctttcctaataaaatgaggaaattgcatcgcattgtctgagtaggtgtcattctattctggggggtggggtggggcaggacagcaagggggaggattgggaagacaatagcaggcatgctggggatgcggtgggctctatgg

SEQ ID NO: 20 - DNA, 2627 bp, synthetic construct
  source 1..2627: mol_type = other DNA
gtgtgtcagttagggtgtggaaagtccccaggctccccagcaggcagaagtatgcaaagcatgcatctcaattagtcagcaaccaggtgtggaaagtccccaggctccccagcaggcagaagtatgcaaagcatgcatctcaattagtcagcaaccatagtcccgcccctaactccgcccatcccgcccctaactccgcccagttccgcccattctccgccccatggctgactaattttttttatttatgcagaggccgaggccgcctcggcctctgagctattccagaagtagtgaggaggcttttttggaggcctaggcttttgcaaaaagctttgcaaagatggataaagttttaaacagagaggaatctttgcagctaatggaccttctaggtcttgaaaggagtgcctgggggaatattcctctgatgagaaaggcatatttaaaaaaatgcaaggagtttcatcctgataaaggaggagatgaagaaaaaatgaagaaaatgaatactctgtacaagaaaatggaagatggagtaaaatatgctcatcaacctgactttggaggcttctgggatgcaactgagattccaacctatggaactgatgaatgggagcagtggtggaatgcctttaatgaggaaaacctgttttgctcagaagaaatgccatctagtgatgatgaggctactgctgactctcaacattctactcctccaaaaaagaagagaaaggtagaagaccccaaggactttccttcagaattgctaagttttttgagtcatgctgtgtttagtaatagaactcttgcttgctttgctatttacaccacaaaggaaaaagctgcactgctatacaagaaaattatggaaaaatattctgtaacctttataagtaggcataacagttataatcataacatactgttttttcttactccacacaggcatagagtgtctgctattaataactatgctcaaaaattgtgtacctttagctttttaatttgtaaaggggttaataaggaatatttgatgtatagtgccttgactagagatccattttctgttattgaggaaagtttgccaggtgggttaaaggagcatgattttaatccagaagaagcagaggaaactaaacaagtgtcctggaagcttgtaacagagtatgcaatggaaacaaaatgtgatgatgtgttgttattgcttgggatgtacttggaatttcagtacagttttgaaatgtgtttaaaatgtattaaaaaagaacagcccagccactataagtaccatgaaaagcattatgcaaatgctgctatatttgctgacagcaaaaaccaaaaaaccatatgccaacaggctgttgatactgttttagctaaaaagcgggttgatagcctacaattaactagagaacaaatgttaacaaacagatttaatgatcttttggataggatggatataatgtttggttctacaggctctgctgacatagaagaatggatggctggagttgcttggctacactgtttgttgcccaaaatggattcagtggtgtatgactttttaaaatgcatggtgtacaacattcctaaaaaaagatactggctgtttaaaggaccaattgatagtggtaaaactacattagcagctgctttgcttgaattatgtggggggaaagctttaaatgttaatttgcccttggacaggctgaactttgagctaggagtagctattgaccagtttttagtagtttttgaggatgtaaagggcactggaggggagtccagagatttgccttcaggtcagggaattaataacctggacaatttaagggattatttggatggcagtgttaaggtaaacttagaaaagaaacacctaaataaaagaactcaaatatttccccctggaatagtcaccatgaatgagtacagtgtgcctaaaacactgcaggccagatttgtaaaacaaatagattttaggcccaaagattatttaaagcattgcctggaacgcagtgagtttttgttagaaaagagaataattcaaagtggcattgctttgcttcttatgttaatttggtacagacctgtggctgagtttgctcaaagtattcagagcagaattgtggagtggaaagagagattggacaaagagtttagtttgtcagtgtatcaaaaaatgaagtttaatgtggctatgggaattggagttttagattggctaagaaacagtgatgatgatgatgaagacagccaggaaaatgctgataaaaatgaagatggtggggagaagaacatggaagactcagggcatgaaacaggcattgattcacagtcccaaggctcatttcaggcccctcagtcctcacagtctgttcatgatcataatcagccataccacatttgtagaggttttacttgctttaaaaaacctcccacacctccccctgaacctgaaacataaaatgaatgcaattgttgttgttaacttgtttattgcagcttataatggttacaaataaagcaatagcatcacaaatttcacaaataaagcatttttttcactgcattctagttgtggtttgtccaaactcatcaatgtatcttatcatgtctggatc

SEQ ID NO: 21 - DNA, 1025 bp, synthetic construct
  source 1..1025: mol_type = other DNA
gtgtgtcagttagggtgtggaaagtccccaggctccccagcaggcagaagtatgcaaagcatgcatctcaattagtcagcaaccaggtgtggaaagtccccaggctccccagcaggcagaagtatgcaaagcatgcatctcaattagtcagcaaccatagtcccgcccctaactccgcccatcccgcccctaactccgcccagttccgcccattctccgccccatggctgactaattttttttatttatgcagaggccgaggccgcctcggcctctgagctattccagaagtagtgaggaggcttttttggaggcctaggcttttgcaaaaagctttgcaaagatggataaagttttaaacagagaggaatctttgcagctaatggaccttctaggtcttgaaaggagtgcctgggggaatattcctctgatgagaaaggcatatttaaaaaaatgcaaggagtttcatcctgataaaggaggagatgaagaaaaaatgaagaaaatgaatactctgtacaagaaaatggaagatggagtaaaatatgctcatcaacctgactttggaggcttctgggatgcaactgaggtatttgcttcttccttaaatcctggtgttgatgcaatgtactgcaaacaatggcctgagtgtgcaaagaaaatgtctgctaactgcatatgcttgctgtgcttactgaggatgaagcatgaaaatagaaaattatacaggaaagatccacttgtgtgggttgattgctactgcttcgattgctttagaatgtggtttggacttgatctttgtgaaggaaccttacttctgtggtgtgacataattggacaaactacctacagagatttaaagctctaaaatgaatgcaattgttgttgttaacttgtttattgcagcttataatggttacaaataaagcaatagcatcacaaatttcacaaataaagcatttttttcactgcattctagttgtggtttgtccaaactcatcaatgtatcttatcatgtctggatc